European Patent Specification EP 3 033 113 B1, published October 4, 2023. Title: A NOVEL PLGA-MODIFIED PEI SELF ASSEMBLY NANOTECHNOLOGY FOR NUCLEIC ACID DRUG DELIVERY. Applicant: Lu, Jian-Ming Yao, Qizhi Chen, Changyi. Application UNKNOWN. The sequence listing filed with the application follows.

SEQUENCE LISTING (3 sequences)

SEQ ID NO: 1 - protein, 23 aa, Artificial Sequence
  Synthetic Peptide
CGGGGDCAWHLGELVWCTGGGGC

SEQ ID NO: 2 - protein, 13 aa, Artificial Sequence
  Synthetic Peptide
DCAWHLGELVWCT

SEQ ID NO: 3 - protein, 36 aa, Artificial Sequence
  Synthetic Peptide
CGGGGDCAWHLGELVWCTDCAWHLGELVWCTGGGGC